European Patent Application EP 4 710 938 A2, published March 18, 2026. Title: IMPROVED VACCINES FOR HUMAN PAPILLOMA VIRUS AND METHODS FOR USING THE SAME. Applicant: The Trustees of The University of Pennsylvania. Application EP, filed March 12, 2014. The sequence listing filed with the application follows.

SEQUENCE LISTING (24 sequences)

SEQ ID NO: 1 - DNA, 873 bp, synthetic construct
  misc_feature 1..873: note = HPV6 E6E7 DNA sequence
  source 1..873: mol_type = other DNA
ggtaccggatccgccaccatggactggacctggattctgttcctggtggccgctgccacacgggtgcacagcgaaagcgccaatgccagcaccagcgctacaaccatcgaccagctgtgcaagaccttcaacctgagcatgcacaccctgcagatcaactgcgtgttctgcaagaacgccctgaccaccgccgagatctacagctacgcctacaagcagctgaaggtgctgttcagaggcggctacccctatgccgcctgcgcctgctgcctggaatttcacggcaagatcaaccagtaccggcacttcgactacgccggctacgccaccaccgtggaagaggaaacaaagcaggacatcctggacgtgctgatccggtgctacctgtgccacaagcccctgtgcgaggtggaaaaagtgaagcacatcctgaccaaggcccggttcatcaagctgaactgcacctggaagggccggtgcctgcactgctggaccacctgtatggaagatatgctgcccagaggccggaagcggcggagccatggcagacacgtgaccctgaaggacatcgtgctggacctgcagccccccgatcctgtgggcctgcactgttacgagcagctggtggacagcagcgaggacgaggtggacgaagtggacggccaggacagccagcccctgaagcagcacttccagatcgtgacctgctgctgcggctgcgacagcaacgtgcggctggtggtgcagtgcaccgagacagacatcagagaggtccagcagctcctgctgggcaccctgaacatcgtgtgccccatctgcgcccccaagacctacccttacgacgtgcccgactacgcctgatgactcgagctc

SEQ ID NO: 2 - protein, 280 aa, synthetic construct
  REGION 1..280: note = HPV6 E6E7 protein sequence
MDWTWILFLVAAATRVHSESANASTSATTIDQLCKTFNLSMHTLQINCVFCKNALTTAEIYSYAYKQLKVLFRGGYPYAACACCLEFHGKINQYRHFDYAGYATTVEEETKQDILDVLIRCYLCHKPLCEVEKVKHILTKARFIKLNCTWKGRCLHCWTTCMEDMLPRGRKRRSHGRHVTLKDIVLDLQPPDPVGLHCYEQLVDSSEDEVDEVDGQDSQPLKQHFQIVTCCCGCDSNVRLVVQCTETDIREVQQLLLGTLNIVCPICAPKTYPYDVPDYA

SEQ ID NO: 3 - DNA, 873 bp, synthetic construct
  misc_feature 1..873: note = HPV11 E6E7 DNA sequence
  source 1..873: mol_type = other DNA
ggtaccggatccgccaccatggactggacctggattctgttcctggtggccgctgccacaagagtgcacagcgagagcaaggatgccagcaccagcgccaccagcatcgaccagctgtgcaagaccttcaacctgagcctgcacaccctgcagatccagtgcgtgttctgccggaacgccctgaccaccgccgagatctacgcctacgcctacaagaacctgaaggtcgtgtggcgggacaacttccccttcgccgcctgcgcctgctgcctggaactgcagggcaagatcaaccagtaccggcacttcaactacgccgcttacgcccccaccgtggaagaggaaacaaacgaggacatcctgaaggtgctgatccggtgctacctgtgccacaagcccctgtgcgagatcgagaagctgaagcacatcctgggcaaggcccggttcatcaagctgaacaaccagtggaagggccggtgcctgcactgctggaccacctgtatggaagatctgctgcccagaggccggaagcggagaagccacggcagactggtcaccctgaaggacatcgtgctggacctgcagccccccgatcctgtgggcctgcactgttacgagcagctggaagatagcagcgaggacgaggtggacaaagtggacaagcaggacgcccagcccctgacccagcactaccagatcctgacctgctgctgcggctgcgacagcaacgtgcggctggtggtggaatgcaccgacggcgacatccggcagctccaggatctgctgctgggcaccctgaacatcgtgtgccccatctgcgcccccaagccctacccctacgacgtgcccgactacgcctgatgactcgagctc

SEQ ID NO: 4 - protein, 280 aa, synthetic construct
  REGION 1..280: note = HPV11 E6E7 protein sequence
MDWTWILFLVAAATRVHSESKDASTSATSIDQLCKTFNLSLHTLQIQCVFCRNALTTAEIYAYAYKNLKVVWRDNFPFAACACCLELQGKINQYRHFNYAAYAPTVEEETNEDILKVLIRCYLCHKPLCEIEKLKHILGKARFIKLNNQWKGRCLHCWTTCMEDLLPRGRKRRSHGRLVTLKDIVLDLQPPDPVGLHCYEQLEDSSEDEVDKVDKQDAQPLTQHYQILTCCCGCDSNVRLVVECTDGDIRQLQDLLLGTLNIVCPICAPKPYPYDVPDYA

SEQ ID NO: 5 - DNA, 828 bp, synthetic construct
  misc_feature 1..828: note = HPV33 E6E7 DNA sequence
  source 1..828: mol_type = other DNA
ggtaccgtcgacggatccgccaccatggactggacctggattctgttcctggtggccgctgctacccgggtgcacagcttccaggacaccgaggaaagcggccggaccctgcacgatctgtgccaggccctggaaaccaccatccacaacatcgagctgcagtgcgtggaatgcaagaagcccctgcagcggagcgaggtgtacgacgccgacctgaccgtggtgtacagagagggcaaccccttcggcatctgcaagctgtgcctgcggttcctgagcaagatcagcgagtaccggcactacaactacagcgtgtacggcaacaccctggaacagaccgtgaagaagcctctgaacgagatcctgatccggtgcatcatctgccagcggcccctgaagcggcacgtggacctgaacaagcggttccacaatatcagcggcagatgggccggcagatgcgccgcctgttggagaagccggcggagagagacagccctgcggggcagaaagcggcggagcagaggccacaagcccaccctgaaagaatacgtgctggacctgtaccccgagcccaccgacctgtacggctacggccagctgagcgacagcagcgacgaggacgagggcctggacagacctgatggacaggcccagcccgccaccgccgactactacatcgtgacctgctgccacacctgtaacaccaccgtgcggctgtgcgtgaacagcaccgccagcgacctgcggacaatccagcagctcctgatgggcaccgtgaacatcgtgtgccctacctgcgcccagctgtgactcgagacgcgtgagctc

SEQ ID NO: 6 - protein, 261 aa, synthetic construct
  REGION 1..261: note = HPV33 E6E7 protein sequence
MDWTWILFLVAAATRVHSFQDTEESGRTLHDLCQALETTIHNIELQCVECKKPLQRSEVYDADLTVVYREGNPFGICKLCLRFLSKISEYRHYNYSVYGNTLEQTVKKPLNEILIRCIICQRPLKRHVDLNKRFHNISGRWAGRCAACWRSRRRETALRGRKRRSRGHKPTLKEYVLDLYPEPTDLYGYGQLSDSSDEDEGLDRPDGQAQPATADYYIVTCCHTCNTTVRLCVNSTASDLRTIQQLLMGTVNIVCPTCAQL

SEQ ID NO: 7 - DNA, 835 bp, synthetic construct
  misc_feature 1..835: note = HPV58 E6E7 DNA sequence
  source 1..835: mol_type = other DNA
ggtaccgtttaaacggatccgccaccatggactggacctggattctgttcctggtggccgctgctacccgggtgcacagcttccaggatgccgaggaaagcggccggaccctgcacgatctgtgccaggccctggaaaccagcgtgcacgagatcgagctgaagtgcgtggaatgcaagaaaaccctgcagcggagcgaggtgtacgacgccgacctgcggatcgtgtaccgggacggcaaccccttcgccgtgtgcaaagtgtgcctgcggctgctgagcaagatcagcgagtaccggcactacaactacagcctgtacggcgacaccctggaacagaccctgaagaagtgcctgaacgagatcctgatccggtgcatcatctgccagcggcccctgaagcggcacgtggacctgaacaagcggttccacaacatcagcggccggtggaccggcagatgcgccgtgtgttggaggcccaggcggagacagacccaggtgcgcggcagaaagcggcggagcagaggcaacaaccccaccctgagagagtacatcctggacctgcaccccgagcccaccgacctgtttggctacggccagctgtgcgacagcagcgacgaggacgagatcggcctggacggccctgatggacaggcccagcccgccaccgccaactactacatcgtgacctgctgctacacctgtggcaccaccgtgcggctgtgcatcaacagcaccaccaccgacgtgcgcaccctgcagcagctcctgatgggcacctgtaccatcgtgtgccccagctgcgcccagcagtgactcgaggcggccgcgagctc

SEQ ID NO: 8 - protein, 262 aa, synthetic construct
  REGION 1..262: note = HPV58 E6E7 protein sequence
MDWTWILFLVAAATRVHSFQDAEESGRTLHDLCQALETSVHEIELKCVECKKTLQRSEVYDADLRIVYRDGNPFAVCKVCLRLLSKISEYRHYNYSLYGDTLEQTLKKCLNEILIRCIICQRPLKRHVDLNKRFHNISGRWTGRCAVCWRPRRRQTQVRGRKRRSRGNNPTLREYILDLHPEPTDLFGYGQLCDSSDEDEIGLDGPDGQAQPATANYYIVTCCYTCGTTVRLCINSTTTDVRTLQQLLMGTCTIVCPSCAQQ

SEQ ID NO: 9 - DNA, 54 bp, synthetic construct
  misc_feature 1..54: note = IgE Leader DNA sequence
  source 1..54: mol_type = other DNA
atggactggacctggatcctgttcctggtggccgctgccacacgggtgcacagc

SEQ ID NO: 10 - protein, 18 aa, synthetic construct
  REGION 1..18: note = IgE leader protein
MDWTWILFLVAAATRVHS

SEQ ID NO: 11 - protein, 15 aa, synthetic construct
  REGION 1..15: note = HPV6 peptide 7
TAEIYSYAYKQLKVL

SEQ ID NO: 12 - protein, 15 aa, synthetic construct
  REGION 1..15: note = HPV11 peptide 7
TAEIYAYAYKNLKVV

SEQ ID NO: 13 - protein, 15 aa, synthetic construct
  REGION 1..15: note = HPV11 peptide 27
HCYEQLEDSSEDEVD

SEQ ID NO: 14 - protein, 15 aa, synthetic construct
  REGION 1..15: note = HPV subdominant peptide 6
FCKNALTTAEIYSYA

SEQ ID NO: 15 - protein, 15 aa, synthetic construct
  REGION 1..15: note = HPV subdominant peptide 9
LFRGGYPYAACACCL

SEQ ID NO: 16 - protein, 15 aa, synthetic construct
  REGION 1..15: note = HPV subdominant peptide 13
YAGYATTVEEETKQD

SEQ ID NO: 17 - DNA, 792 bp, synthetic construct
  misc_feature 1..792: note = pGX3005 insert HPV31 E6/E7 DNA sequence
  source 1..792: mol_type = other DNA
atggactggacatggattctgttcctggtcgccgccgcaactagagtgcattcattcaaaaaccccgccgagtctgggagaaaactgcacgagctgagctccgcactggagatcccctacgatgaactgaggctgaactgcgtgtattgtaaaggacagctgactgagaccgaagtgctggacactgatctgaccattgtctaccgagacgatacaccttatggcgtgtgcactaaatgtctgcgcttctactcaaaggtgagcgagtttagatggtacaggtatagcgtctatggcaccacactggaaaaactgacaaacaaggggatctgcgacctgctgatcaggtgcattacttgtcagcgccctctgcagcgacacctggataagaagaagcggttccataatatcggcgggcggtggaccgggagatgcatcgtgtgctggcggagaccacggacagagactcaggtccgagggcggaaaaggcgctctagaggagaaaccccaacactgcaggactacgtgctggatctgcagcccgaggccacagacctgcatggatatggccagctgcccgactctagtgatgaggaagacgtgatcgatagtcccgccggccaggctaagcctgatacctccaactacaatattgtcacattttgctgtcagtgcgaatccactctgaggctgtgcgtgcagtctacccaggtcgacatccgcattctgcaggaactgctgatgggatctttcggaatcgtgtgccctaattgctccaccagactgtgataa

SEQ ID NO: 18 - protein, 262 aa, synthetic construct
  REGION 1..262: note = pGX3005 insert HPV31 E6/E7 protein sequence
MDWTWILFLVAAATRVHSFKNPAESGRKLHELSSALEIPYDELRLNCVYCKGQLTETEVLDTDLTIVYRDDTPYGVCTKCLRFYSKVSEFRWYRYSVYGTTLEKLTNKGICDLLIRCITCQRPLQRHLDKKKRFHNIGGRWTGRCIVCWRRPRTETQVRGRKRRSRGETPTLQDYVLDLQPEATDLHGYGQLPDSSDEEDVIDSPAGQAKPDTSNYNIVTFCCQCESTLRLCVQSTQVDIRILQELLMGSFGIVCPNCSTRL

SEQ ID NO: 19 - DNA, 792 bp, synthetic construct
  misc_feature 1..792: note = pGX3007 insert HPV52 E6/E7 DNA sequence
  source 1..792: mol_type = other DNA
atggactggacctggattctgttcctggtggctgctgctacacgggtgcattcatttgaagaccctgctacatctggacgaactctgcacgagctgtgcgaagtgctggaggaatctgtccatgagatcaggctgcagtgcgtgcagtgtaagaaagagctgcagcggagagaagtgtacaagaccgacctgcggattgtctacagagataacaatccctatggagtgtgcatcatgtgcctgcggttcctgtctaaaattagtgaatacagacactaccagtattccctgtatggcaagacactggaggaacgagtgcggaaaccactgtctgagatcaccattcgctgcatcatttgtcagacacccctggaacgacacgtcaacgcaaacaagcggttccataacatcatgggaaggtggactggccgctgcagtgagtgttggagaccaaggcctgtgacccaggtccgcggacgaaaacggcggagccggggcgacaaggcaaccatcaaagactacattctggatctgcagcctgagaccacagatctgcatggctatgggcagctgggggacagctccgatgaggaagacacagatggggtggacagaccagatggacaggccgaacaggctacaagcaattactatatcgtcacttattgccactcatgtgacagcactctgaggctgtgcattcattccactgctaccgatctgcgcacactgcagcagatgctgctgggaacactgcaggtggtctgtccaggatgtgcccgactgtgataa

SEQ ID NO: 20 - protein, 262 aa, synthetic construct
  REGION 1..262: note = pGX3007 insert HPV52 E6/E7 protein sequence
MDWTWILFLVAAATRVHSFEDPATSGRTLHELCEVLEESVHEIRLQCVQCKKELQRREVYKTDLRIVYRDNNPYGVCIMCLRFLSKISEYRHYQYSLYGKTLEERVRKPLSEITIRCIICQTPLERHVNANKRFHNIMGRWTGRCSECWRPRPVTQVRGRKRRSRGDKATIKDYILDLQPETTDLHGYGQLGDSSDEEDTDGVDRPDGQAEQATSNYYIVTYCHSCDSTLRLCIHSTATDLRTLQQMLLGTLQVVCPGCARL

SEQ ID NO: 21 - DNA, 818 bp, synthetic construct
  misc_feature 1..818: note = HPV genotype 16 E6-E7 DNA sequence
  source 1..818: mol_type = other DNA
gaattcgccaccatggactggacctggatcctgttcctggtggccgccgccacacgggtgcacagcttccaggacccccaggagagcggcagaaagctgcctcagctgtgtaccgagctgcagaccaccatccacgacatcatcctggagtgtgtgtactgtaagcagcagctgctgaggagagaggtgtacgaccgggacctgtgtatcgtgtacagggacggcaatccctacgccgtgtgtgacaagtgcctgaagttctacagcaagatcagcgagtaccggcactactgctacagcctgtacggcaccaccctggagcagcagtacaacaagcccctgtgtgacctgctgatccggtgtatcaactgccagaagcccctgcagagacacctggacaagaagcagcggttccacaacatcaggggcagatggaccggcagatgtatgagctgctgccggagcagcagaaccagaagggagacccagctgagaggccggaagagaagaagccacggcgatacccccaccctgcacgagtacatgctggacctgcagcctgagaccaccgatctgtacggctacggccagctgaatgacagcagcgaggaggaggatgagatcgacggccctgccggccaggccgagcccgacagagcccactacaacatcgtgaccttttgctgtaagtgtgacagcaccctgagactgtgcgtgcagagcacccacgtggacatcagaaccctggaggatctgctgatgggcaccctgggcatcgtgtgtcccatctgctcccagaaaccctgatgagcggccgc

SEQ ID NO: 22 - protein, 264 aa, synthetic construct
  REGION 1..264: note = HPV genotype 16 E6-E7 protein sequence
MDWTWILFLVAAATRVHSFQDPQESGRKLPQLCTELQTTIHDIILECVYCKQQLLRREVYDRDLCIVYRDGNPYAVCDKCLKFYSKISEYRHYCYSLYGTTLEQQYNKPLCDLLIRCINCQKPLQRHLDKKQRFHNIRGRWTGRCMSCCRSSRTRRETQLRGRKRRSHGDTPTLHEYMLDLQPETTDLYGYGQLNDSSEEEDEIDGPAGQAEPDRAHYNIVTFCCKCDSTLRLCVQSTHVDIRTLEDLLMGTLGIVCPICSQKP

SEQ ID NO: 23 - DNA, 837 bp, synthetic construct
  misc_feature 1..837: note = HPV genotype 18 E6-E7 DNA sequence
  source 1..837: mol_type = other DNA
atggactggacctggatcctgttcctggtggccgctgccacacgggtgcacagcgccagattcgaggaccccaccaggagcggctacaagctgcccgatctgtgtaccgagctgaacaccagcctgcaggacatcgagatcacctgtgtgtactgtaagaccgtgctggagctgaccgaggtgttcgagaaggacctgttcgtggtgtacagggacagcatcccccacgccgcctgccacaagtgtatcgacttctacagccggatccgggagctgagacactacagcgacagcgtgtacggcgataccctggagaagctgaccaacaccggcctgtacaacctgctgatccggtgcctgagatgccagaagcccctgctgagacacctgaacgagaagcggcggttccacaacatcgccggccactacagaggccagtgccacagctgctgtaacagggccaggcaggagagactgcagcggagaagagagacccaggtgaggggcaggaagagaagaagccacggccccaaggccaccctgcaggatatcgtgctgcacctggagccccagaatgagatccccgtggatctgctgggccacggccagctgtccgacagcgaggaggagaacgacgagatcgacggcgtgaatcaccagcacctgcctgccagaagagccgagcctcagaggcacaccatgctgtgtatgtgctgtaagtgtgaggcccggatcgaactggtggtggagagcagcgccgacgacctgagagccttccagcagctgttcctgaacaccctgagcttcgtgtgtccttggtgtgccagccagcagtga

SEQ ID NO: 24 - protein, 278 aa, synthetic construct
  REGION 1..278: note = HPV genotype 18 E6-E7 protein sequence
MDWTWILFLVAAATRVHSARFEDPTRSGYKLPDLCTELNTSLQDIEITCVYCKTVLELTEVFEKDLFVVYRDSIPHAACHKCIDFYSRIRELRHYSDSVYGDTLEKLTNTGLYNLLIRCLRCQKPLLRHLNEKRRFHNIAGHYRGQCHSCCNRARQERLQRRRETQVRGRKRRSHGPKATLQDIVLHLEPQNEIPVDLLGHGQLSDSEEENDEIDGVNHQHLPARRAEPQRHTMLCMCCKCEARIELVVESSADDLRAFQQLFLNTLSFVCPWCASQQ